European Patent Application EP 4 609 878 A1, published September 3, 2025. Title: Production method of radioactive pharmaceutical composition. Applicant: 日本メジフィジックス株式会社. The sequence listing filed with the application follows.

SEQUENCE LISTING (15 sequences)

SEQ ID NO: 1 - protein, 13 aa, synthetic construct
  REGION 1..13: note = antibody modifying peptide
  SITE 6: note = misc_feature - lysine, cystein, aspartic acid, glutamic acid, 2-aminosuberic acid, or diaminopropionic acid
DCAYHXGELVWCT

SEQ ID NO: 2 - protein, 17 aa, synthetic construct
  REGION 1..17: note = antibody modifying peptide
  SITE 8: note = misc_feature - lysine, cystein, aspartic acid, glutamic acid, 2-aminosuberic acid, or diaminopropionic acid
GPDCAYHXGELVWCTFH

SEQ ID NO: 3 - protein, 13 aa, synthetic construct
  REGION 1..13: note = antibody modifying peptide
  SITE 6: note = misc_feature - lysine, cystein, aspartic acid, glutamic acid, 2-aminosuberic acid, or diaminopropionic acid
RCAYHXGELVWCS

SEQ ID NO: 4 - protein, 17 aa, synthetic construct
  REGION 1..17: note = antibody modifying peptide
  SITE 8: note = misc_feature - lysine, cystein, aspartic acid, glutamic acid, 2-aminosuberic acid, or diaminopropionic acid
GPRCAYHXGELVWCSFH

SEQ ID NO: 5 - protein, 17 aa, synthetic construct
  REGION 1..17: note = antibody modifying peptide
  SITE 8: note = misc_feature - lysine, cystein, aspartic acid, glutamic acid, 2-aminosuberic acid, or diaminopropionic acid
SPDCAYHXGELVWCTFH

SEQ ID NO: 6 - protein, 17 aa, synthetic construct
  REGION 1..17: note = antibody modifying peptide
  SITE 8: note = misc_feature -lysine, cystein, aspartic acid, glutamic acid, 2-aminosuberic acid, or diaminopropionic acid
GDDCAYHXGELVWCTFH

SEQ ID NO: 7 - protein, 17 aa, synthetic construct
  REGION 1..17: note = antibody modifying peptide
  SITE 8: note = misc_feature - lysine, cystein, aspartic acid, glutamic acid, 2-aminosuberic acid, or diaminopropionic acid
GPSCAYHXGELVWCTFH

SEQ ID NO: 8 - protein, 17 aa, synthetic construct
  REGION 1..17: note = antibody modifying peptide
  SITE 8: note = misc_feature - lysine, cystein, aspartic acid, glutamic acid, 2-aminosuberic acid, or diaminopropionic acid
GPDCAYHXGELVWCSFH

SEQ ID NO: 9 - protein, 17 aa, synthetic construct
  REGION 1..17: note = antibody modifying peptide
  SITE 8: note = misc_feature - lysine, cystein, aspartic acid, glutamic acid, 2-aminosuberic acid, or diaminopropionic acid
GPDCAYHXGELVWCTHH

SEQ ID NO: 10 - protein, 17 aa, synthetic construct
  REGION 1..17: note = antibody modifying peptide
  SITE 8: note = misc_feature - lysine, cystein, aspartic acid, glutamic acid, 2-aminosuberic acid, or diaminopropionic acid
GPDCAYHXGELVWCTFY

SEQ ID NO: 11 - protein, 17 aa, synthetic construct
  REGION 1..17: note = antibody modifying peptide
  SITE 8: note = misc_feature -lysine, cystein, aspartic acid, glutamic acid, 2-aminosuberic acid, or diaminopropionic acid
SPDCAYHXGELVWCTFY

SEQ ID NO: 12 - protein, 17 aa, synthetic construct
  REGION 1..17: note = antibody modifying peptide
  SITE 8: note = misc_feature - lysine, cystein, aspartic acid, glutamic acid, 2-aminosuberic acid, or diaminopropionic acid
SDDCAYHXGELVWCTFY

SEQ ID NO: 13 - protein, 17 aa, synthetic construct
  REGION 1..17: note = antibody modifying peptide
  SITE 8: note = misc_feature - lysine, cystein, aspartic acid, glutamic acid, 2-aminosuberic acid, or diaminopropionic acid
RGNCAYHXGQLVWCTYH

SEQ ID NO: 14 - protein, 17 aa, synthetic construct
  REGION 1..17: note = antibody modifying peptide
  SITE 2: note = misc_feature - homocysteine
  SITE 8: note = misc_feature - lysine, cystein, aspartic acid, glutamic acid, 2-aminosuberic acid, or diaminopropionic acid
  SITE 16: note = misc_feature - homocysteine
GXDCAYHXGELVWCTXH

SEQ ID NO: 15 - protein, 17 aa, synthetic construct
  DISULFID 4..14: note = Cys-Cys
GPDCAYHKGELVWCTFH